European Patent Application EP 4 378 955 A1, published June 5, 2024. Title: 一种抗DLL3抗体及其制备方法、其药物偶联物和应用. Applicant: 上海复旦张江生物医药股份有限公司. Application WO PCT/CN2022/109050, filed July 29, 2022. The sequence listing filed with the application follows.

SEQUENCE LISTING (114 sequences)

SEQ ID NO: 1 - protein, 214 aa, synthetic construct
EIVMTQSPATLSVSPGERATLSCKASQSVSNDVVWYQQKPGQAPRLLIYYASNRYTGIPARFSGSGSGTEFTLTISSLQSEDFAVYYCQQDYTSPWTFGQGTKLEIKRTVAAPSVFIFPPSDEQLKSGTASVVCLLNNFYPREAKVQWKVDNALQSGNSQESVTEQDSKDSTYSLSSTLTLSKADYEKHKVYACEVTHQGLSSPVTKSFNRGEC

SEQ ID NO: 2 - protein, 447 aa, synthetic construct
QVQLVQSGAEVKKPGASVKVSCKASGYTFTNYGMNWVRQAPGQGLEWMGWINTYTGEPTYADDFKGRVTMTTDTSTSTAYMELRSLRSDDTAVYYCARIGDSSPSDYWGQGTLVTVSSASTKGPSVFPLAPSSKSTSGGTAALGCLVKDYFPEPVTVSWNSGALTSGVHTFPAVLQSSGLYSLSSVVTVPSSSLGTQTYICNVNHKPSNTKVDKKVEPKSCDKTHTCPPCPAPELLGGPSVFLFPPKPKDTLMISRTPEVTCVVVDVSHEDPEVKFNWYVDGVEVHNAKTKPREEQYNSTYRVVSVLTVLHQDWLNGKEYKCKVSNKALPAPIEKTISKAKGQPREPQVYTLPPSRDELTKNQVSLTCLVKGFYPSDIAVEWESNGQPENNYKTTPPVLDSDGSFFLYSKLTVDKSRWQQGNVFSCSVMHEALHNHYTQKSLSLSPG

SEQ ID NO: 3 - protein, 214 aa, synthetic construct
AIQLTQSPSSLSASVGDRVTITCRASENIYYNLAWYQQKPGKAPKLLIYTANSLEDGVPSRFSGSGSGTDFTLTISSLQPEDFATYFCKQAYDVPPTFGGGTKLEIKRTVAAPSVFIFPPSDEQLKSGTASVVCLLNNFYPREAKVQWKVDNALQSGNSQESVTEQDSKDSTYSLSSTLTLSKADYEKHKVYACEVTHQGLSSPVTKSFNRGEC

SEQ ID NO: 4 - protein, 447 aa, synthetic construct
QVQLVQSGAEVKKPGASVKVSCKASGYTFTRYWIHWIRQAPGQGLEWMGYINPTTVYTEFNQNFKDRVTMTRDTSTSTVYMELSSLRSEDTAVYYCARGGSNFFDYWGQGTTVTVSSASTKGPSVFPLAPSSKSTSGGTAALGCLVKDYFPEPVTVSWNSGALTSGVHTFPAVLQSSGLYSLSSVVTVPSSSLGTQTYICNVNHKPSNTKVDKRVEPKSCDKTHTCPPCPAPELLGGPSVFLFPPKPKDTLMISRTPEVTCVVVDVSHEDPEVKFNWYVDGVEVHNAKTKPREEQYNSTYRVVSVLTVLHQDWLNGKEYKCKVSNKALPAPIEKTISKAKGQPREPQVYTLPPSREEMTKNQVSLTCLVKGFYPSDIAVEWESNGQPENNYKTTPPVLDSDGSFFLYSKLTVDKSRWQQGNVFSCSVMHEALHNHYTQKSLSLSPGK

SEQ ID NO: 5 - protein, 389 aa, synthetic construct
  REGION 1..16: note = V5 label; note (original language) = V5标签
  REGION 334..389: note = Intracellular sequence; note (original language) = 胞内序列
GKPIPNPLLGLDSTSGARCEPPAVGTACTRLCRPRSAPSRCGPGLRPCAPLEDECEAPLVCRAGCSPEHGFCEQPGECRCLEGWTGPLCTVPVSTSSCLSPRGPSSATTGCLVPGPGPCDGNPCANGGSCSETPRSFECTCPRGFYGLRCEVSGVTCADGPCFNGGLCVGGADPDSAYICHCPPGFQGSNCEKRVDRCSLQPCRNGGLCLDLGHALRCRCRAGFAGPRCEHDLDDCAGRACANGGTCVEGGGAHRCSCALGFGGRDCRERADPCAARPCAHGGRCYAHFSGLVCACAPGYMGARCEFPVHPDGASALPAAPPGLRPGDPQRYLSGGGGSGAGVIAVIVVVVIAIVAGIVVLVISRKKRMAKYEKAEIKEMGEMHRELNA

SEQ ID NO: 6 - protein, 349 aa, synthetic construct
  REGION 1..16: note = V5 label; note (original language) = V5标签
  REGION 294..349: note = Intracellular sequence; note (original language) = 胞内序列
GKPIPNPLLGLDSTSGAPLVCRAGCSPEHGFCEQPGECRCLEGWTGPLCTVPVSTSSCLSPRGPSSATTGCLVPGPGPCDGNPCANGGSCSETPRSFECTCPRGFYGLRCEVSGVTCADGPCFNGGLCVGGADPDSAYICHCPPGFQGSNCEKRVDRCSLQPCRNGGLCLDLGHALRCRCRAGFAGPRCEHDLDDCAGRACANGGTCVEGGGAHRCSCALGFGGRDCRERADPCAARPCAHGGRCYAHFSGLVCACAPGYMGARCEFPVHPDGASALPAAPPGLRPGDPQRYLSGGGGSGAGVIAVIVVVVIAIVAGIVVLVISRKKRMAKYEKAEIKEMGEMHRELNA

SEQ ID NO: 7 - protein, 291 aa, synthetic construct
  REGION 1..16: note = V5 label; note (original language) = V5标签
  REGION 236..291: note = Intracellular sequence; note (original language) = 胞内序列
GKPIPNPLLGLDSTSGGPGPCDGNPCANGGSCSETPRSFECTCPRGFYGLRCEVSGVTCADGPCFNGGLCVGGADPDSAYICHCPPGFQGSNCEKRVDRCSLQPCRNGGLCLDLGHALRCRCRAGFAGPRCEHDLDDCAGRACANGGTCVEGGGAHRCSCALGFGGRDCRERADPCAARPCAHGGRCYAHFSGLVCACAPGYMGARCEFPVHPDGASALPAAPPGLRPGDPQRYLSGGGGSGAGVIAVIVVVVIAIVAGIVVLVISRKKRMAKYEKAEIKEMGEMHRELNA

SEQ ID NO: 8 - protein, 253 aa, synthetic construct
  REGION 1..16: note = V5 label; note (original language) = V5标签
  REGION 198..253: note = Intracellular sequence; note (original language) = 胞内序列
GKPIPNPLLGLDSTSGSGVTCADGPCFNGGLCVGGADPDSAYICHCPPGFQGSNCEKRVDRCSLQPCRNGGLCLDLGHALRCRCRAGFAGPRCEHDLDDCAGRACANGGTCVEGGGAHRCSCALGFGGRDCRERADPCAARPCAHGGRCYAHFSGLVCACAPGYMGARCEFPVHPDGASALPAAPPGLRPGDPQRYLSGGGGSGAGVIAVIVVVVIAIVAGIVVLVISRKKRMAKYEKAEIKEMGEMHRELNA

SEQ ID NO: 9 - protein, 8 aa, synthetic construct
GYTFTESA

SEQ ID NO: 10 - protein, 8 aa, synthetic construct
INPNNGGI

SEQ ID NO: 11 - protein, 11 aa, synthetic construct
GSSYYRDYFDY

SEQ ID NO: 12 - protein, 7 aa, synthetic construct
ENVGTYV

SEQ ID NO: 13 - protein, 118 aa, synthetic construct
EVQLQQSGPELVKPGASVKISCKASGYTFTDYNMNWVKQSQGKSLEWIGYIYPYNGGTGYNQKFKTKATLTVDNSSSTAYMEFRSLTSEDSAVYYCARSDPYYTMDYWGQGTSVTVSS

SEQ ID NO: 14 - protein, 9 aa, synthetic construct
GQSYSYPLT

SEQ ID NO: 15 - protein, 118 aa, synthetic construct
EVQLQQSGPELVKPGASVKISCKTSGYTFTESAMHWVKQSHGKSLEWIGGINPNNGGISYSQKFKGKATLTVDKSSSTAYMELRSLTSEDSAVYYCGSSYYRDYFDYWGQGTTLTVSS

SEQ ID NO: 16 - protein, 107 aa, synthetic construct
NIVMTQSPESMSMSVGERVTLSCKASENVGTYVSWYQQKPDQSPKLLIYGASNRYTGVPDRFTGSGSATHFTLTISSVQAEDLADYHCGQSYSYPLTFGAGTKLELK

SEQ ID NO: 17 - protein, 447 aa, synthetic construct
  REGION 1..447: note = 1A5 HC
EVQLQQSGPELVKPGASVKISCKTSGYTFTESAMHWVKQSHGKSLEWIGGINPNNGGISYSQKFKGKATLTVDKSSSTAYMELRSLTSEDSAVYYCGSSYYRDYFDYWGQGTTLTVSSASTKGPSVFPLAPSSKSTSGGTAALGCLVKDYFPEPVTVSWNSGALTSGVHTFPAVLQSSGLYSLSSVVTVPSSSLGTQTYICNVNHKPSNTKVDKKVEPKSCDKTHTCPPCPAPELLGGPSVFLFPPKPKDTLMISRTPEVTCVVVDVSHEDPEVKFNWYVDGVEVHNAKTKPREEQYNSTYRVVSVLTVLHQDWLNGKEYKCKVSNKALPAPIEKTISKAKGQPREPQVYTLPPSRDELTKNQVSLTCLVKGFYPSDIAVEWESNGQPENNYKTTPPVLDSDGSFFLYSKLTVDKSRWQQGNVFSCSVMHEALHNHYTQKSLSLSPG

SEQ ID NO: 18 - protein, 214 aa, synthetic construct
NIVMTQSPESMSMSVGERVTLSCKASENVGTYVSWYQQKPDQSPKLLIYGASNRYTGVPDRFTGSGSATHFTLTISSVQAEDLADYHCGQSYSYPLTFGAGTKLELKRTVAAPSVFIFPPSDEQLKSGTASVVCLLNNFYPREAKVQWKVDNALQSGNSQESVTEQDSKDSTYSLSSTLTLSKADYEKHKVYACEVTHQGLSSPVTKSFNRGEC

SEQ ID NO: 19 - protein, 8 aa, synthetic construct
GYTFTENT

SEQ ID NO: 20 - protein, 8 aa, synthetic construct
INPRNGVT

SEQ ID NO: 21 - protein, 11 aa, synthetic construct
TNTYYRDYFDY

SEQ ID NO: 22 - protein, 117 aa, synthetic construct
EVQLQQSGPELEKPGASVRISCKASGYSFTDYNMHWVKQSNGKSLEWIGNIDPYYGGTNYNQKFEGKATLTVDKSSSTAYMQLKSLTSEDSAVYYCARGGNNYGDYWGQGTTLTVSS

SEQ ID NO: 23 - protein, 107 aa, synthetic construct
DIQMTQSPASLAASVGETVTITCRASENIYYSLAWYQQKQGKSPQLLIFNANSLEDGVPSRFSGSGSGTQYSMKINSMQPEDTATYFCKQAYDVPWTFGGGTKLEIK

SEQ ID NO: 24 - protein, 9 aa, synthetic construct
GQTYTYPLT

SEQ ID NO: 25 - protein, 118 aa, synthetic construct
EVQLQQSGPELVKPGASVKISCKTSGYTFTENTMHWVKQSHGESLEWIGGINPRNGVTSYNQKFKGKATLTVDKSSSTAYMELRSLTSEDSAVYYCTNTYYRDYFDYWGQGTTLTVSS

SEQ ID NO: 26 - protein, 107 aa, synthetic construct
NIVMTQSPKSMSMSVGERVTLSCKASENVGTYVSWYQQKPDQSPKLLIYGASNRYTGVPDRFTGSGSPTDFTLTISRMQAEDLAHYYCGQTYTYPLTFGAGTKLELK

SEQ ID NO: 27 - protein, 447 aa, synthetic construct
EVQLQQSGPELVKPGASVKISCKTSGYTFTENTMHWVKQSHGESLEWIGGINPRNGVTSYNQKFKGKATLTVDKSSSTAYMELRSLTSEDSAVYYCTNTYYRDYFDYWGQGTTLTVSSASTKGPSVFPLAPSSKSTSGGTAALGCLVKDYFPEPVTVSWNSGALTSGVHTFPAVLQSSGLYSLSSVVTVPSSSLGTQTYICNVNHKPSNTKVDKKVEPKSCDKTHTCPPCPAPELLGGPSVFLFPPKPKDTLMISRTPEVTCVVVDVSHEDPEVKFNWYVDGVEVHNAKTKPREEQYNSTYRVVSVLTVLHQDWLNGKEYKCKVSNKALPAPIEKTISKAKGQPREPQVYTLPPSRDELTKNQVSLTCLVKGFYPSDIAVEWESNGQPENNYKTTPPVLDSDGSFFLYSKLTVDKSRWQQGNVFSCSVMHEALHNHYTQKSLSLSPG

SEQ ID NO: 28 - protein, 214 aa, synthetic construct
NIVMTQSPKSMSMSVGERVTLSCKASENVGTYVSWYQQKPDQSPKLLIYGASNRYTGVPDRFTGSGSPTDFTLTISRMQAEDLAHYYCGQTYTYPLTFGAGTKLELKRTVAAPSVFIFPPSDEQLKSGTASVVCLLNNFYPREAKVQWKVDNALQSGNSQESVTEQDSKDSTYSLSSTLTLSKADYEKHKVYACEVTHQGLSSPVTKSFNRGEC

SEQ ID NO: 29 - protein, 8 aa, synthetic construct
GYTFTDYA

SEQ ID NO: 30 - protein, 9 aa, synthetic construct
IVSTDSGKT

SEQ ID NO: 31 - protein, 15 aa, synthetic construct
ARNPYYDYDGYAMDY

SEQ ID NO: 32 - protein, 6 aa, synthetic construct
DHINNW

SEQ ID NO: 33 - protein, 107 aa, synthetic construct
IIVMTQTPKFLLVSAGDRVTISCKASQSVNNDVAWYQQKPGQSPKLLIYFTSNRFTGVPDRFTGSGYGTDFTFTISSVQAEDLAVYFCQQDHNSPYTFGGGTKLEIK

SEQ ID NO: 34 - protein, 9 aa, synthetic construct
QQYWSIPYT

SEQ ID NO: 35 - protein, 122 aa, synthetic construct
QVQLQQSGPELVRPGVSVKISCKGSGYTFTDYAIHWVKQSRAKSPEWIGIVSTDSGKTSFNQKFKGKATMTVDKSSTTAYMELVRLTSEDSAIYYCARNPYYDYDGYAMDYWGQGTSVTVSS

SEQ ID NO: 36 - protein, 107 aa, synthetic construct
DIQMTQSSSYLSVSLGGRVTIICKASDHINNWLAWYQQKPGNAPRLIISGATSLETGVPSRFSGSGSGKDYTLSITSLQTEDVATYYCQQYWSIPYTFGGGTKLEIK

SEQ ID NO: 37 - protein, 451 aa, synthetic construct
QVQLQQSGPELVRPGVSVKISCKGSGYTFTDYAIHWVKQSRAKSPEWIGIVSTDSGKTSFNQKFKGKATMTVDKSSTTAYMELVRLTSEDSAIYYCARNPYYDYDGYAMDYWGQGTSVTVSSASTKGPSVFPLAPSSKSTSGGTAALGCLVKDYFPEPVTVSWNSGALTSGVHTFPAVLQSSGLYSLSSVVTVPSSSLGTQTYICNVNHKPSNTKVDKKVEPKSCDKTHTCPPCPAPELLGGPSVFLFPPKPKDTLMISRTPEVTCVVVDVSHEDPEVKFNWYVDGVEVHNAKTKPREEQYNSTYRVVSVLTVLHQDWLNGKEYKCKVSNKALPAPIEKTISKAKGQPREPQVYTLPPSRDELTKNQVSLTCLVKGFYPSDIAVEWESNGQPENNYKTTPPVLDSDGSFFLYSKLTVDKSRWQQGNVFSCSVMHEALHNHYTQKSLSLSPG

SEQ ID NO: 38 - protein, 214 aa, synthetic construct
DIQMTQSSSYLSVSLGGRVTIICKASDHINNWLAWYQQKPGNAPRLIISGATSLETGVPSRFSGSGSGKDYTLSITSLQTEDVATYYCQQYWSIPYTFGGGTKLEIKRTVAAPSVFIFPPSDEQLKSGTASVVCLLNNFYPREAKVQWKVDNALQSGNSQESVTEQDSKDSTYSLSSTLTLSKADYEKHKVYACEVTHQGLSSPVTKSFNRGEC

SEQ ID NO: 39 - protein, 10 aa, synthetic construct
GFSLSTSGMG

SEQ ID NO: 40 - protein, 7 aa, synthetic construct
IWWDDVK

SEQ ID NO: 41 - protein, 18 aa, synthetic construct
ARIAEVTGQVGLHYAMDY

SEQ ID NO: 42 - protein, 7 aa, synthetic construct
SSVNSSS

SEQ ID NO: 43 - protein, 447 aa, synthetic construct
EVQLQQSGPELVKPGASVKISCKASGYTFTDYNMNWVKQSQGKSLEWIGYIYPYNGGTGYNQKFKTKATLTVDNSSSTAYMEFRSLTSEDSAVYYCARSDPYYTMDYWGQGTSVTVSSASTKGPSVFPLAPSSKSTSGGTAALGCLVKDYFPEPVTVSWNSGALTSGVHTFPAVLQSSGLYSLSSVVTVPSSSLGTQTYICNVNHKPSNTKVDKKVEPKSCDKTHTCPPCPAPELLGGPSVFLFPPKPKDTLMISRTPEVTCVVVDVSHEDPEVKFNWYVDGVEVHNAKTKPREEQYNSTYRVVSVLTVLHQDWLNGKEYKCKVSNKALPAPIEKTISKAKGQPREPQVYTLPPSRDELTKNQVSLTCLVKGFYPSDIAVEWESNGQPENNYKTTPPVLDSDGSFFLYSKLTVDKSRWQQGNVFSCSVMHEALHNHYTQKSLSLSPG

SEQ ID NO: 44 - protein, 9 aa, synthetic construct
HQFHRSPFT

SEQ ID NO: 45 - protein, 126 aa, synthetic construct
QVTLKESGPGILQPSQTLSLTCSFSGFSLSTSGMGVGWIRQPSGKGLEWLALIWWDDVKRYHPALKSRLTISKDTSSSQVFLKIASVDTADTATYYCARIAEVTGQVGLHYAMDYWGQGTSVTVSS

SEQ ID NO: 46 - protein, 108 aa, synthetic construct
QTVLTQSPAIMSASLGERVTMTCTASSSVNSSSLHWYQQKPGSSPKLWIYTTSNLASGVPARFSGSGSGTSYSLTISSMEAEDAATYYCHQFHRSPFTFGSGTKLEIK

SEQ ID NO: 47 - protein, 455 aa, synthetic construct
QVTLKESGPGILQPSQTLSLTCSFSGFSLSTSGMGVGWIRQPSGKGLEWLALIWWDDVKRYHPALKSRLTISKDTSSSQVFLKIASVDTADTATYYCARIAEVTGQVGLHYAMDYWGQGTSVTVSSASTKGPSVFPLAPSSKSTSGGTAALGCLVKDYFPEPVTVSWNSGALTSGVHTFPAVLQSSGLYSLSSVVTVPSSSLGTQTYICNVNHKPSNTKVDKKVEPKSCDKTHTCPPCPAPELLGGPSVFLFPPKPKDTLMISRTPEVTCVVVDVSHEDPEVKFNWYVDGVEVHNAKTKPREEQYNSTYRVVSVLTVLHQDWLNGKEYKCKVSNKALPAPIEKTISKAKGQPREPQVYTLPPSRDELTKNQVSLTCLVKGFYPSDIAVEWESNGQPENNYKTTPPVLDSDGSFFLYSKLTVDKSRWQQGNVFSCSVMHEALHNHYTQKSLSLSPG

SEQ ID NO: 48 - protein, 215 aa, synthetic construct
  REGION 1..215: note = 32E8 LC
QTVLTQSPAIMSASLGERVTMTCTASSSVNSSSLHWYQQKPGSSPKLWIYTTSNLASGVPARFSGSGSGTSYSLTISSMEAEDAATYYCHQFHRSPFTFGSGTKLEIKRTVAAPSVFIFPPSDEQLKSGTASVVCLLNNFYPREAKVQWKVDNALQSGNSQESVTEQDSKDSTYSLSSTLTLSKADYEKHKVYACEVTHQGLSSPVTKSFNRGEC

SEQ ID NO: 49 - protein, 8 aa, synthetic construct
GFAFSSYD

SEQ ID NO: 50 - protein, 8 aa, synthetic construct
ISSGGSYT

SEQ ID NO: 51 - protein, 11 aa, synthetic construct
ASPLLGLRFAY

SEQ ID NO: 52 - protein, 9 aa, synthetic construct
TGAVTTINY

SEQ ID NO: 53 - protein, 214 aa, synthetic construct
IIVMTQTPKFLLVSAGDRVTISCKASQSVNNDVAWYQQKPGQSPKLLIYFTSNRFTGVPDRFTGSGYGTDFTFTISSVQAEDLAVYFCQQDHNSPYTFGGGTKLEIKRTVAAPSVFIFPPSDEQLKSGTASVVCLLNNFYPREAKVQWKVDNALQSGNSQESVTEQDSKDSTYSLSSTLTLSKADYEKHKVYACEVTHQGLSSPVTKSFNRGEC

SEQ ID NO: 54 - protein, 9 aa, synthetic construct
ALYYSNHWV

SEQ ID NO: 55 - protein, 118 aa, synthetic construct
EVKLVESGGGLVKPGGSLKLSCAASGFAFSSYDMSWVRQTPEKRLEWVATISSGGSYTYYPDSVKGRFTISRDNGRNTLYLQMSSLRSEDTALYYCASPLLGLRFAYWGQGTLVTVSA

SEQ ID NO: 56 - protein, 109 aa
QAVVTQESALTTSPGETVTLTCRSSTGAVTTINYANWVQEKPDHLFTGLIGGTNNRAPGVPARFSGSLIGDKAALTITGAQTEDEAIYFCALYYSNHWVFGGGTKLTVL

SEQ ID NO: 57 - protein, 447 aa, synthetic construct
EVKLVESGGGLVKPGGSLKLSCAASGFAFSSYDMSWVRQTPEKRLEWVATISSGGSYTYYPDSVKGRFTISRDNGRNTLYLQMSSLRSEDTALYYCASPLLGLRFAYWGQGTLVTVSAASTKGPSVFPLAPSSKSTSGGTAALGCLVKDYFPEPVTVSWNSGALTSGVHTFPAVLQSSGLYSLSSVVTVPSSSLGTQTYICNVNHKPSNTKVDKKVEPKSCDKTHTCPPCPAPELLGGPSVFLFPPKPKDTLMISRTPEVTCVVVDVSHEDPEVKFNWYVDGVEVHNAKTKPREEQYNSTYRVVSVLTVLHQDWLNGKEYKCKVSNKALPAPIEKTISKAKGQPREPQVYTLPPSRDELTKNQVSLTCLVKGFYPSDIAVEWESNGQPENNYKTTPPVLDSDGSFFLYSKLTVDKSRWQQGNVFSCSVMHEALHNHYTQKSLSLSPG

SEQ ID NO: 58 - protein, 216 aa, synthetic construct
QAVVTQESALTTSPGETVTLTCRSSTGAVTTINYANWVQEKPDHLFTGLIGGTNNRAPGVPARFSGSLIGDKAALTITGAQTEDEAIYFCALYYSNHWVFGGGTKLTVLRTVAAPSVFIFPPSDEQLKSGTASVVCLLNNFYPREAKVQWKVDNALQSGNSQESVTEQDSKDSTYSLSSTLTLSKADYEKHKVYACEVTHQGLSSPVTKSFNRGEC

SEQ ID NO: 59 - protein, 9 aa, synthetic construct
GYTFTYYVM

SEQ ID NO: 60 - protein, 8 aa, synthetic construct
INPYNDGT

SEQ ID NO: 61 - protein, 12 aa, synthetic construct
ARWLLREYAMDY

SEQ ID NO: 62 - protein, 6 aa, synthetic construct
DNIHNY

SEQ ID NO: 63 - protein, 8 aa, synthetic construct
GYSFTDYN

SEQ ID NO: 64 - protein, 9 aa, synthetic construct
QHFWSTPWT

SEQ ID NO: 65 - protein, 119 aa, synthetic construct
EVQLQQSGPELVRPGASVRMSCKASGYTFTYYVMHWVKQKPGLGLEWIGYINPYNDGTEYNEKFKGKATLTSDKSSSTAFMELSSLTSEDSAVYYCARWLLREYAMDYWGQGTSVTVSS

SEQ ID NO: 66 - protein, 107 aa, synthetic construct
DIQMTQSPASLSASVGETVTITCRASDNIHNYLAWYQQKQGKSPQLLVYNAKTLADGVPSRFSGSGSGTQYSLKINSLQPEDFGSYYCQHFWSTPWTFGGGTKLEIK

SEQ ID NO: 67 - protein, 448 aa, synthetic construct
EVQLQQSGPELVRPGASVRMSCKASGYTFTYYVMHWVKQKPGLGLEWIGYINPYNDGTEYNEKFKGKATLTSDKSSSTAFMELSSLTSEDSAVYYCARWLLREYAMDYWGQGTSVTVSSASTKGPSVFPLAPSSKSTSGGTAALGCLVKDYFPEPVTVSWNSGALTSGVHTFPAVLQSSGLYSLSSVVTVPSSSLGTQTYICNVNHKPSNTKVDKKVEPKSCDKTHTCPPCPAPELLGGPSVFLFPPKPKDTLMISRTPEVTCVVVDVSHEDPEVKFNWYVDGVEVHNAKTKPREEQYNSTYRVVSVLTVLHQDWLNGKEYKCKVSNKALPAPIEKTISKAKGQPREPQVYTLPPSRDELTKNQVSLTCLVKGFYPSDIAVEWESNGQPENNYKTTPPVLDSDGSFFLYSKLTVDKSRWQQGNVFSCSVMHEALHNHYTQKSLSLSPG

SEQ ID NO: 68 - protein, 214 aa, synthetic construct
DIQMTQSPASLSASVGETVTITCRASDNIHNYLAWYQQKQGKSPQLLVYNAKTLADGVPSRFSGSGSGTQYSLKINSLQPEDFGSYYCQHFWSTPWTFGGGTKLEIKRTVAAPSVFIFPPSDEQLKSGTASVVCLLNNFYPREAKVQWKVDNALQSGNSQESVTEQDSKDSTYSLSSTLTLSKADYEKHKVYACEVTHQGLSSPVTKSFNRGEC

SEQ ID NO: 69 - protein, 8 aa, synthetic construct
GYTFTTYV

SEQ ID NO: 70 - protein, 8 aa, synthetic construct
INPYNDDT

SEQ ID NO: 71 - protein, 16 aa, synthetic construct
ARWGLTGTGDYYAMDY

SEQ ID NO: 72 - protein, 6 aa, synthetic construct
GNVHNY

SEQ ID NO: 73 - protein, 446 aa, synthetic construct
EVQLQQSGPELEKPGASVRISCKASGYSFTDYNMHWVKQSNGKSLEWIGNIDPYYGGTNYNQKFEGKATLTVDKSSSTAYMQLKSLTSEDSAVYYCARGGNNYGDYWGQGTTLTVSSASTKGPSVFPLAPSSKSTSGGTAALGCLVKDYFPEPVTVSWNSGALTSGVHTFPAVLQSSGLYSLSSVVTVPSSSLGTQTYICNVNHKPSNTKVDKKVEPKSCDKTHTCPPCPAPELLGGPSVFLFPPKPKDTLMISRTPEVTCVVVDVSHEDPEVKFNWYVDGVEVHNAKTKPREEQYNSTYRVVSVLTVLHQDWLNGKEYKCKVSNKALPAPIEKTISKAKGQPREPQVYTLPPSRDELTKNQVSLTCLVKGFYPSDIAVEWESNGQPENNYKTTPPVLDSDGSFFLYSKLTVDKSRWQQGNVFSCSVMHEALHNHYTQKSLSLSPG

SEQ ID NO: 74 - protein, 9 aa, synthetic construct
QHFWTTPWT

SEQ ID NO: 75 - protein, 123 aa, synthetic construct
EVQLQQSGPELVKPGASVKMSCKASGYTFTTYVMHWVKQKPGQGLEWIGYINPYNDDTNYNEKFKGKATLTSDKSSSTAYMELSSLTSEDSAVYYCARWGLTGTGDYYAMDYWGQGTSVTVSS

SEQ ID NO: 76 - protein, 107 aa, synthetic construct
DIQMTQSPASLSASVGETVTITCRASGNVHNYLAWYQQKQGRSPQVLVYNAKTLADGVPSRFSGSGSGTQYSLKINSLLPEDFGSYYCQHFWTTPWTFGGGTTLEIK

SEQ ID NO: 77 - protein, 452 aa, synthetic construct
EVQLQQSGPELVKPGASVKMSCKASGYTFTTYVMHWVKQKPGQGLEWIGYINPYNDDTNYNEKFKGKATLTSDKSSSTAYMELSSLTSEDSAVYYCARWGLTGTGDYYAMDYWGQGTSVTVSSASTKGPSVFPLAPSSKSTSGGTAALGCLVKDYFPEPVTVSWNSGALTSGVHTFPAVLQSSGLYSLSSVVTVPSSSLGTQTYICNVNHKPSNTKVDKKVEPKSCDKTHTCPPCPAPELLGGPSVFLFPPKPKDTLMISRTPEVTCVVVDVSHEDPEVKFNWYVDGVEVHNAKTKPREEQYNSTYRVVSVLTVLHQDWLNGKEYKCKVSNKALPAPIEKTISKAKGQPREPQVYTLPPSRDELTKNQVSLTCLVKGFYPSDIAVEWESNGQPENNYKTTPPVLDSDGSFFLYSKLTVDKSRWQQGNVFSCSVMHEALHNHYTQKSLSLSPG

SEQ ID NO: 78 - protein, 214 aa, synthetic construct
DIQMTQSPASLSASVGETVTITCRASGNVHNYLAWYQQKQGRSPQVLVYNAKTLADGVPSRFSGSGSGTQYSLKINSLLPEDFGSYYCQHFWTTPWTFGGGTTLEIKRTVAAPSVFIFPPSDEQLKSGTASVVCLLNNFYPREAKVQWKVDNALQSGNSQESVTEQDSKDSTYSLSSTLTLSKADYEKHKVYACEVTHQGLSSPVTKSFNRGEC

SEQ ID NO: 79 - protein, 7 aa, synthetic construct
FTFSNYT

SEQ ID NO: 80 - protein, 8 aa, synthetic construct
FSSGGSYT

SEQ ID NO: 81 - protein, 17 aa, synthetic construct
SRDRRSDGYYHLYAMDY

SEQ ID NO: 82 - protein, 6 aa, synthetic construct
QDISHY

SEQ ID NO: 83 - protein, 8 aa, synthetic construct
IDPYYGGT

SEQ ID NO: 84 - protein, 9 aa, synthetic construct
QQGYTLPLT

SEQ ID NO: 85 - protein, 124 aa, synthetic construct
DVKLVESGGGLVKPGGSLKLSCAASGFTFSNYTISWVRQTPEKRLEWVATFSSGGSYTYYSDSVKGRFTISRDNAKNTLYLQMSSLKSEDTAMYYCSRDRRSDGYYHLYAMDYWGQGTSVTVSS

SEQ ID NO: 86 - protein, 107 aa, synthetic construct
DIQMTQTTSSLSASLGDRVTISCRASQDISHYLNWYQQKPDGTVKLLIYYTSRLHSGVPSRFSGSGSGTAYSLTISNLEQEDIATYFCQQGYTLPLTFGAGTKLELK

SEQ ID NO: 87 - protein, 453 aa, synthetic construct
DVKLVESGGGLVKPGGSLKLSCAASGFTFSNYTISWVRQTPEKRLEWVATFSSGGSYTYYSDSVKGRFTISRDNAKNTLYLQMSSLKSEDTAMYYCSRDRRSDGYYHLYAMDYWGQGTSVTVSSASTKGPSVFPLAPSSKSTSGGTAALGCLVKDYFPEPVTVSWNSGALTSGVHTFPAVLQSSGLYSLSSVVTVPSSSLGTQTYICNVNHKPSNTKVDKKVEPKSCDKTHTCPPCPAPELLGGPSVFLFPPKPKDTLMISRTPEVTCVVVDVSHEDPEVKFNWYVDGVEVHNAKTKPREEQYNSTYRVVSVLTVLHQDWLNGKEYKCKVSNKALPAPIEKTISKAKGQPREPQVYTLPPSRDELTKNQVSLTCLVKGFYPSDIAVEWESNGQPENNYKTTPPVLDSDGSFFLYSKLTVDKSRWQQGNVFSCSVMHEALHNHYTQKSLSLSPG

SEQ ID NO: 88 - protein, 214 aa, synthetic construct
DIQMTQTTSSLSASLGDRVTISCRASQDISHYLNWYQQKPDGTVKLLIYYTSRLHSGVPSRFSGSGSGTAYSLTISNLEQEDIATYFCQQGYTLPLTFGAGTKLELKRTVAAPSVFIFPPSDEQLKSGTASVVCLLNNFYPREAKVQWKVDNALQSGNSQESVTEQDSKDSTYSLSSTLTLSKADYEKHKVYACEVTHQGLSSPVTKSFNRGEC

SEQ ID NO: 89 - protein, 8 aa, synthetic construct
GYTFTDYN

SEQ ID NO: 90 - protein, 8 aa, synthetic construct
IYPFNGGI

SEQ ID NO: 91 - protein, 8 aa, synthetic construct
ARLNWEGY

SEQ ID NO: 92 - protein, 6 aa, synthetic construct
QDINSY

SEQ ID NO: 93 - protein, 10 aa, synthetic construct
ARGGNNYGDY

SEQ ID NO: 94 - protein, 9 aa, synthetic construct
LQYAEFPYT

SEQ ID NO: 95 - protein, 115 aa, synthetic construct
EVQFQQSGPELVKPGASVKISCKASGYTFTDYNIHWVRQSQGKSLEWIGLIYPFNGGIVYNQKFKSKATLTVDNSSTSAYMELRSLSSEDSAVYFCARLNWEGYWGQGSTLIVSS

SEQ ID NO: 96 - protein, 107 aa, synthetic construct
DIKMTQSPSSIYAFLGERVTITCKASQDINSYLSWFQQKPGKSPKTLIYRANRLVGGVPSRFSGSGSGQDYSLTISSLEYEDVGDYYCLQYAEFPYTFGGGTKLEIK

SEQ ID NO: 97 - protein, 444 aa, synthetic construct
EVQFQQSGPELVKPGASVKISCKASGYTFTDYNIHWVRQSQGKSLEWIGLIYPFNGGIVYNQKFKSKATLTVDNSSTSAYMELRSLSSEDSAVYFCARLNWEGYWGQGSTLIVSSASTKGPSVFPLAPSSKSTSGGTAALGCLVKDYFPEPVTVSWNSGALTSGVHTFPAVLQSSGLYSLSSVVTVPSSSLGTQTYICNVNHKPSNTKVDKKVEPKSCDKTHTCPPCPAPELLGGPSVFLFPPKPKDTLMISRTPEVTCVVVDVSHEDPEVKFNWYVDGVEVHNAKTKPREEQYNSTYRVVSVLTVLHQDWLNGKEYKCKVSNKALPAPIEKTISKAKGQPREPQVYTLPPSRDELTKNQVSLTCLVKGFYPSDIAVEWESNGQPENNYKTTPPVLDSDGSFFLYSKLTVDKSRWQQGNVFSCSVMHEALHNHYTQKSLSLSPG

SEQ ID NO: 98 - protein, 214 aa, synthetic construct
DIKMTQSPSSIYAFLGERVTITCKASQDINSYLSWFQQKPGKSPKTLIYRANRLVGGVPSRFSGSGSGQDYSLTISSLEYEDVGDYYCLQYAEFPYTFGGGTKLEIKRTVAAPSVFIFPPSDEQLKSGTASVVCLLNNFYPREAKVQWKVDNALQSGNSQESVTEQDSKDSTYSLSSTLTLSKADYEKHKVYACEVTHQGLSSPVTKSFNRGEC

SEQ ID NO: 99 - protein, 8 aa, synthetic construct
GFNFKDYY

SEQ ID NO: 100 - protein, 8 aa, synthetic construct
IDPENGNA

SEQ ID NO: 101 - protein, 11 aa, synthetic construct
ASEDAYYPFAY

SEQ ID NO: 102 - protein, 12 aa, synthetic construct
QSLLYSSNQKNY

SEQ ID NO: 103 - protein, 6 aa, synthetic construct
ENIYYS

SEQ ID NO: 104 - protein, 8 aa, synthetic construct
QQYYSYRT

SEQ ID NO: 105 - protein, 118 aa, synthetic construct
EVQLQQSGAELVRPGALVKLSCKASGFNFKDYYIHWVKQRPELGLEWIGWIDPENGNAIYDPKFQDKASITADTSSNTAYLHLSSLTSEGTAVYYCASEDAYYPFAYWGQGTLVTVSS

SEQ ID NO: 106 - protein, 112 aa, synthetic construct
DIVMSQSPSSLAVSVGEKVTMRCKSSQSLLYSSNQKNYLAWYQQKPGQSPKLLIYWASTRESGVPDRFTGSGSGTDFTLTISSVKAEDLAVYFCQQYYSYRTFGGGTKLEIK

SEQ ID NO: 107 - protein, 446 aa, synthetic construct
EVQLQQSGAELVRPGALVKLSCKASGFNFKDYYIHWVKQRPELGLEWIGWIDPENGNAIYDPKFQDKASITADTSSNTAYLHLSSLTSEGTAVYYCASEDAYYPFAYWGQGTLVTVSASTKGPSVFPLAPSSKSTSGGTAALGCLVKDYFPEPVTVSWNSGALTSGVHTFPAVLQSSGLYSLSSVVTVPSSSLGTQTYICNVNHKPSNTKVDKKVEPKSCDKTHTCPPCPAPELLGGPSVFLFPPKPKDTLMISRTPEVTCVVVDVSHEDPEVKFNWYVDGVEVHNAKTKPREEQYNSTYRVVSVLTVLHQDWLNGKEYKCKVSNKALPAPIEKTISKAKGQPREPQVYTLPPSRDELTKNQVSLTCLVKGFYPSDIAVEWESNGQPENNYKTTPPVLDSDGSFFLYSKLTVDKSRWQQGNVFSCSVMHEALHNHYTQKSLSLSPG

SEQ ID NO: 108 - protein, 219 aa, synthetic construct
DIVMSQSPSSLAVSVGEKVTMRCKSSQSLLYSSNQKNYLAWYQQKPGQSPKLLIYWASTRESGVPDRFTGSGSGTDFTLTISSVKAEDLAVYFCQQYYSYRTFGGGTKLEIKRTVAAPSVFIFPPSDEQLKSGTASVVCLLNNFYPREAKVQWKVDNALQSGNSQESVTEQDSKDSTYSLSSTLTLSKADYEKHKVYACEVTHQGLSSPVTKSFNRGEC

SEQ ID NO: 109 - protein, 214 aa, synthetic construct
DIQMTQSPASLAASVGETVTITCRASENIYYSLAWYQQKQGKSPQLLIFNANSLEDGVPSRFSGSGSGTQYSMKINSMQPEDTATYFCKQAYDVPWTFGGGTKLEIKRTVAAPSVFIFPPSDEQLKSGTASVVCLLNNFYPREAKVQWKVDNALQSGNSQESVTEQDSKDSTYSLSSTLTLSKADYEKHKVYACEVTHQGLSSPVTKSFNRGEC

SEQ ID NO: 110 - protein, 8 aa, synthetic construct
IYPYNGGT

SEQ ID NO: 111 - protein, 11 aa, synthetic construct
ARSDPYYTMDY

SEQ ID NO: 112 - protein, 6 aa, synthetic construct
QSVNND

SEQ ID NO: 113 - protein, 12 aa, synthetic construct
NANKQAYDVPWT

SEQ ID NO: 114 - protein, 9 aa, synthetic construct
QQDHNSPYT